European Patent Specification EP 3 397 965 B1, published September 11, 2024. Title: Compositions and methods for assessing the risk of cancer occurrence. Applicant: Syncerus S.à r.l. The sequence listing filed with the application follows.

SEQUENCE LISTING (39 sequences)

SEQ ID NO: 1 - protein, 80 aa, Homo sapiens
  SITE (1)..(80): Human progastrin
SWKPRSQQPDAPLGTGANRDLELPWLEQQGPASHHRRQLGPQGPPHLVADPSKKQGPWLEEEEEAYGWMDFGRRSAEDEN

SEQ ID NO: 2 - protein, 14 aa, Artificial
  Amino acids 1-14, N-terminal extremity of human progastrin
SWKPRSQQPDAPLG

SEQ ID NO: 3 - protein, 26 aa, Artificial
  Amino acids 55-80, C-terminal extremity of human progastrin
QGPWLEEEEEAYGWMDFGRRSAEDEN

SEQ ID NO: 4 - protein, 8 aa, Artificial
  6B5B11C10 CDR-H1
GYIFTSYW

SEQ ID NO: 5 - protein, 8 aa, Artificial
  6B5B11C10 CDR-H2
FYPGNSDS

SEQ ID NO: 6 - protein, 8 aa, Artificial
  6B5B11C10 CDR-H3
TRRDSPQY

SEQ ID NO: 7 - protein, 11 aa, Artificial
  6B5B11C10 CDR-L1
QSIVHSNGNTY

SEQ ID NO: 8 - protein, 3 aa, Artificial
  6B5B11C10 CDR-L2
KVS

SEQ ID NO: 9 - protein, 9 aa, Artificial
  6B5B11C10 CDR-L3
FQGSHVPFT

SEQ ID NO: 10 - protein, 7 aa, Artificial
  20D2C3G2 CDR-H1
GYTFSSW

SEQ ID NO: 11 - protein, 8 aa, Artificial
  20D2C3G2 CDR-H2
FLPGSGST

SEQ ID NO: 12 - protein, 11 aa, Artificial
  20D2C3G2 CDR-H3
ATDGNYDWFAY

SEQ ID NO: 13 - protein, 11 aa, Artificial
  20D2C3G2 CDR-L1
QSLVHSSGVTY

SEQ ID NO: 14 - protein, 3 aa, Artificial
  20D2C3G2 CDR-L2
KVS

SEQ ID NO: 15 - protein, 9 aa, Artificial
  20D2C3G2 CDR-L3
SQSTHVPPT

SEQ ID NO: 16 - protein, 8 aa, Artificial
  1E9D9B6 CDR-H1
GYTFTSYY

SEQ ID NO: 17 - protein, 8 aa, Artificial
  1E9D9B6 CDR-H2
INPSNGGT

SEQ ID NO: 18 - protein, 10 aa, Artificial
  1E9D9B6 CDR-H3
TRGGYYPFDY

SEQ ID NO: 19 - protein, 11 aa, Artificial
  1E9D9B6 CDR-L1
QSLLDSDGKTY

SEQ ID NO: 20 - protein, 3 aa, Artificial
  1E9D9B6 CDR-L2
LVS

SEQ ID NO: 21 - protein, 9 aa, Artificial
  1E9D9B6 CDR-L3
WQGTHSPYT

SEQ ID NO: 22 - protein, 9 aa, Artificial
  1B3B4F11 CDR-H1
GYSITSDYA

SEQ ID NO: 23 - protein, 7 aa, Artificial
  1B3B4F11 CDR-H2
ISFSGYT

SEQ ID NO: 24 - protein, 14 aa, Artificial
  1B3B4F11 CDR-H3
AREVNYGDSYHFDY

SEQ ID NO: 25 - protein, 7 aa, Artificial
  1B3B4F11 CDR-L1
SQHRTYT

SEQ ID NO: 26 - protein, 7 aa, Artificial
  1B3B4F11 CDR-L2
VKKDGSH

SEQ ID NO: 27 - protein, 13 aa, Artificial
  1B3B4F11 CDR-L3
GVGDAIKGQSVFV

SEQ ID NO: 28 - protein, 8 aa, Artificial
  1C10D3B9 CDR-H1
GFTFTTYA

SEQ ID NO: 29 - protein, 8 aa, Artificial
  1C10D3B9 CDR-H2
ISSGGTYT

SEQ ID NO: 30 - protein, 10 aa, Artificial
  1C10D3B9 CDR-H3
ATQGNYSLDF

SEQ ID NO: 31 - protein, 11 aa, Artificial
  1C10D3B9 CDR-L1
KSLRHTKGITF

SEQ ID NO: 32 - protein, 3 aa, Artificial
  1C10D3B9 CDR-L2
QMS

SEQ ID NO: 33 - protein, 9 aa, Artificial
  1C10D3B9 CDR-L3
AQNLELPLT

SEQ ID NO: 34 - protein, 8 aa, Artificial
  2C6C3C7 CDR-H1
GFIFSSYG

SEQ ID NO: 35 - protein, 8 aa, Artificial
  2C6C3C7 CDR-H2
INTFGDRT

SEQ ID NO: 36 - protein, 7 aa, Artificial
  2C6C3C7 CDR-H3
ARGTGTY

SEQ ID NO: 37 - protein, 11 aa, Artificial
  2C6C3C7 CDR-L1
QSLLDSDGKTY

SEQ ID NO: 38 - protein, 3 aa, Artificial
  2C6C3C7 CDR-L2
LVS

SEQ ID NO: 39 - protein, 9 aa, Artificial
  2C6C3C7 CDR-L3
WQGTHFPQT